European Patent Application EP 4 582 442 A2, published July 9, 2025. Title: TNFR2 antagonists with improved stability. Applicant: University Stuttgart. Application EP. The sequence listing filed with the application follows.

SEQUENCE LISTING (108 sequences)

SEQ ID NO: 1-2 - skipped (2 entries)

SEQ ID NO: 3 - protein, 6 aa, Homo sapiens
VYFGII

SEQ ID NO: 4 - protein, 5 aa, Homo sapiens
PVAHV

SEQ ID NO: 5 - protein, 233 aa, Homo sapiens
MSTESMIRDVELAEEALPKKTGGPQGSRRCLFLSLFSFLIVAGATTLFCLLHFGVIGPQREEFPRDLSLISPLAQAVRSSSRTPSDKPVAHVVANPQAEGQLQWLNRRANALLANGVELRDNQLVVPSEGLYLIYSQVLFKGQGCPSTHVLLTHTISRIAVSYQTKVNLLSAIKSPCQRETPEGAEAKPWYEPIYLGGVFQLEKGDRLSAEINRPDYLDFAESGQVYFGIIAL

SEQ ID NO: 6 - protein, 4 aa, Homo sapiens
PSDK

SEQ ID NO: 7 - protein, 5 aa, Homo sapiens
TPSDK

SEQ ID NO: 8 - protein, 6 aa, Homo sapiens
RTPSDK

SEQ ID NO: 9 - protein, 7 aa, Homo sapiens
SRTPSDK

SEQ ID NO: 10 - protein, 8 aa, Homo sapiens
SSRTPSDK

SEQ ID NO: 11 - protein, 4 aa, Homo sapiens
HSTK

SEQ ID NO: 12 - protein, 5 aa, Homo sapiens
AHSTK

SEQ ID NO: 13 - protein, 6 aa, Homo sapiens
LAHSTK

SEQ ID NO: 14 - protein, 7 aa, Homo sapiens
HLAHSTK

SEQ ID NO: 15 - protein, 8 aa, Homo sapiens
LHLAHSTK

SEQ ID NO: 16 - protein, 4 aa, synthetic construct
  REGION 1..4: note = linker
GGGG

SEQ ID NO: 17 - protein, 4 aa, synthetic construct
  REGION 1..4: note = linker
GGGS

SEQ ID NO: 18 - protein, 4 aa, synthetic construct
  REGION 1..4: note = linker
GGSG

SEQ ID NO: 19 - protein, 4 aa, synthetic construct
  REGION 1..4: note = linker
GSGG

SEQ ID NO: 20 - protein, 4 aa, synthetic construct
  REGION 1..4: note = linker
SGGG

SEQ ID NO: 21 - protein, 5 aa, synthetic construct
  REGION 1..5: note = linker
GGGGG

SEQ ID NO: 22 - protein, 5 aa, synthetic construct
  REGION 1..5: note = linker
SGGGG

SEQ ID NO: 23 - protein, 5 aa, synthetic construct
  REGION 1..5: note = linker
GSGGG

SEQ ID NO: 24 - protein, 5 aa, synthetic construct
  REGION 1..5: note = linker
GGSGG

SEQ ID NO: 25 - protein, 5 aa, synthetic construct
  REGION 1..5: note = linker
GGGSG

SEQ ID NO: 26 - protein, 5 aa, synthetic construct
  REGION 1..5: note = linker
GGGGS

SEQ ID NO: 27 - protein, 6 aa, synthetic construct
  REGION 1..6: note = linker
GGGGGG

SEQ ID NO: 28 - protein, 6 aa, synthetic construct
  REGION 1..6: note = linker
SGGGGG

SEQ ID NO: 29 - protein, 6 aa, synthetic construct
  REGION 1..6: note = linker
GSGGGG

SEQ ID NO: 30 - protein, 6 aa, synthetic construct
  REGION 1..6: note = linker
GGSGGG

SEQ ID NO: 31 - protein, 6 aa, synthetic construct
  REGION 1..6: note = linker
GGGSGG

SEQ ID NO: 32 - protein, 6 aa, synthetic construct
  REGION 1..6: note = linker
GGGGSG

SEQ ID NO: 33 - protein, 6 aa, synthetic construct
  REGION 1..6: note = linker
GGGGGS

SEQ ID NO: 34 - protein, 8 aa, synthetic construct
  REGION 1..8: note = linker
GGGSGGGS

SEQ ID NO: 35 - protein, 8 aa, synthetic construct
  REGION 1..8: note = linker
SGGGSGGG

SEQ ID NO: 36 - protein, 8 aa, synthetic construct
  REGION 1..8: note = linker
GGGGGGGG

SEQ ID NO: 37 - protein, 8 aa, synthetic construct
  REGION 1..8: note = linker
GSGGGSGG

SEQ ID NO: 38 - protein, 8 aa, synthetic construct
  REGION 1..8: note = linker
GGSGGGSG

SEQ ID NO: 39 - protein, 9 aa, synthetic construct
  REGION 1..9: note = linker
SGGGSGGGS

SEQ ID NO: 40 - protein, 9 aa, synthetic construct
  REGION 1..9: note = linker
GSGGGSGGG

SEQ ID NO: 41 - protein, 9 aa, synthetic construct
  REGION 1..9: note = linker
GGSGGGSGG

SEQ ID NO: 42 - protein, 9 aa, synthetic construct
  REGION 1..9: note = linker
GGGSGGGSG

SEQ ID NO: 43 - protein, 10 aa, synthetic construct
  REGION 1..10: note = linker
SGGGSGGGSG

SEQ ID NO: 44 - protein, 10 aa, synthetic construct
  REGION 1..10: note = linker
GSGGGSGGGS

SEQ ID NO: 45 - protein, 10 aa, synthetic construct
  REGION 1..10: note = linker
GGSGGGSGGG

SEQ ID NO: 46 - protein, 10 aa, synthetic construct
  REGION 1..10: note = linker
GGGSGGGSGG

SEQ ID NO: 47 - protein, 11 aa, synthetic construct
  REGION 1..11: note = linker
SGGGSGGGSGG

SEQ ID NO: 48 - protein, 11 aa, synthetic construct
  REGION 1..11: note = lnker
GSGGGSGGGSG

SEQ ID NO: 49 - protein, 11 aa, synthetic construct
  REGION 1..11: note = linker
GGSGGGSGGGS

SEQ ID NO: 50 - protein, 11 aa, synthetic construct
  REGION 1..11: note = linker
GGGSGGGSGGG

SEQ ID NO: 51 - protein, 9 aa, Homo sapiens
SSSRTPSDK

SEQ ID NO: 52 - protein, 10 aa, Homo sapiens
RSSSRTPSDK

SEQ ID NO: 53 - protein, 12 aa, synthetic construct
  REGION 1..12: note = linker
GGGSGGGSGGGS

SEQ ID NO: 54 - protein, 16 aa, synthetic construct
  REGION 1..16: note = linker
GGGSGGGSGGGSGGGS

SEQ ID NO: 55 - protein, 205 aa, Homo sapiens
MTPPERLFLPRVCGTTLHLLLLGLLLVLLPGAQGLPGVGLTPSAAQTARQHPKMHLAHSTLKPAAHLIGDPSKQNSLLWRANTDRAFLQDGFSLSNNSLLVPTSGIYFVYSQVVFSGKAYSPKATSSPLYLAHEVQLFSSQYPFHVPLLSSQKMVYPGLQEPWLHSMYHGAAFQLTQGDQLSTHTDGIPHLVLSPSTVFFGAFAL

SEQ ID NO: 56 - protein, 6 aa, Homo sapiens
VFFGAF

SEQ ID NO: 57 - protein, 5 aa, Homo sapiens
PAAHL

SEQ ID NO: 58 - protein, 23 aa, synthetic construct
  REGION 1..23: note = scTNFR2 construct
GIIALGGGGSSSRTPSDKPVAHV

SEQ ID NO: 59 - protein, 18 aa, synthetic construct
  REGION 1..18: note = scTNFR2 construct
GIIALSSRTPSDKPVAHV

SEQ ID NO: 60 - protein, 16 aa, synthetic construct
  REGION 1..16: note = scTNFR2 contruct
GIIALRTPSDKPVAHV

SEQ ID NO: 61 - protein, 14 aa, synthetic construct
  REGION 1..14: note = scTNFR2 construct
GIIALPSDKPVAHV

SEQ ID NO: 62 - protein, 17 aa, synthetic construct
  REGION 1..17: note = scTNFR2 construct
GIIALGGGGSDKPVAHV

SEQ ID NO: 63 - protein, 12 aa, synthetic construct
  REGION 1..12: note = scTNFR2 construct
GIIALDKPVAHV

SEQ ID NO: 64 - protein, 18 aa, synthetic construct
  REGION 1..18: note = scTNFR2 construct
GIIALGGGSGGGSPVAHV

SEQ ID NO: 65 - protein, 507 aa, synthetic construct
  REGION 1..507: note = scTNFR2 (118)
METDTLLLWVLLLWVPGSTGMCGSHHHHHHSGIPASSRTPSDKPVAHVVANPQAEGQLQWLNRRANALLANGVELRDNQLVVPSEGLYLIYSQVLFKGQGCPSTHVLLTHTISRIAVSYQTKVNLLSAIKSPCQRETPEGAEAKPWYEPIYLGGVFQLEKGDRLSAEINRPDYLNFRESGQVYFGIIALGGGGSSSRTPSDKPVAHVVANPQAEGQLQWLNRRANALLANGVELRDNQLVVPSEGLYLIYSQVLFKGQGCPSTHVLLTHTISRIAVSYQTKVNLLSAIKSPCQRETPEGAEAKPWYEPIYLGGVFQLEKGDRLSAEINRPDYLNFRESGQVYFGIIALGGGGSSSRTPSDKPVAHVVANPQAEGQLQWLNRRANALLANGVELRDNQLVVPSEGLYLIYSQVLFKGQGCPSTHVLLTHTISRIAVSYQTKVNLLSAIKSPCQRETPEGAEAKPWYEPIYLGGVFQLEKGDRLSAEINRPDYLNFRESGQVYFGIIAL

SEQ ID NO: 66 - protein, 497 aa, synthetic construct
  REGION 1..497: note = scTNFR2 (127)
METDTLLLWVLLLWVPGSTGMCGSHHHHHHSGIPASSRTPSDKPVAHVVANPQAEGQLQWLNRRANALLANGVELRDNQLVVPSEGLYLIYSQVLFKGQGCPSTHVLLTHTISRIAVSYQTKVNLLSAIKSPCQRETPEGAEAKPWYEPIYLGGVFQLEKGDRLSAEINRPDYLNFRESGQVYFGIIALSSRTPSDKPVAHVVANPQAEGQLQWLNRRANALLANGVELRDNQLVVPSEGLYLIYSQVLFKGQGCPSTHVLLTHTISRIAVSYQTKVNLLSAIKSPCQRETPEGAEAKPWYEPIYLGGVFQLEKGDRLSAEINRPDYLNFRESGQVYFGIIALSSRTPSDKPVAHVVANPQAEGQLQWLNRRANALLANGVELRDNQLVVPSEGLYLIYSQVLFKGQGCPSTHVLLTHTISRIAVSYQTKVNLLSAIKSPCQRETPEGAEAKPWYEPIYLGGVFQLEKGDRLSAEINRPDYLNFRESGQVYFGIIAL

SEQ ID NO: 67 - protein, 485 aa, synthetic construct
  REGION 1..485: note = scTNFR2 (129)
METDTLLLWVLLLWVPGSTGMCGSHHHHHHSGIPAPSDKPVAHVVANPQAEGQLQWLNRRANALLANGVELRDNQLVVPSEGLYLIYSQVLFKGQGCPSTHVLLTHTISRIAVSYQTKVNLLSAIKSPCQRETPEGAEAKPWYEPIYLGGVFQLEKGDRLSAEINRPDYLNFRESGQVYFGIIALPSDKPVAHVVANPQAEGQLQWLNRRANALLANGVELRDNQLVVPSEGLYLIYSQVLFKGQGCPSTHVLLTHTISRIAVSYQTKVNLLSAIKSPCQRETPEGAEAKPWYEPIYLGGVFQLEKGDRLSAEINRPDYLNFRESGQVYFGIIALPSDKPVAHVVANPQAEGQLQWLNRRANALLANGVELRDNQLVVPSEGLYLIYSQVLFKGQGCPSTHVLLTHTISRIAVSYQTKVNLLSAIKSPCQRETPEGAEAKPWYEPIYLGGVFQLEKGDRLSAEINRPDYLNFRESGQVYFGIIAL

SEQ ID NO: 68 - protein, 490 aa, synthetic construct
  REGION 1..490: note = scTNFR2 (139)
METDTLLLWVLLLWVPGSTGMCGSHHHHHHSGIPASDKPVAHVVANPQAEGQLQWLNRRANALLANGVELRDNQLVVPSEGLYLIYSQVLFKGQGCPSTHVLLTHTISRIAVSYQTKVNLLSAIKSPCQRETPEGAEAKPWYEPIYLGGVFQLEKGDRLSAEINRPDYLNFRESGQVYFGIIALGGGGSDKPVAHVVANPQAEGQLQWLNRRANALLANGVELRDNQLVVPSEGLYLIYSQVLFKGQGCPSTHVLLTHTISRIAVSYQTKVNLLSAIKSPCQRETPEGAEAKPWYEPIYLGGVFQLEKGDRLSAEINRPDYLNFRESGQVYFGIIALGGGGSDKPVAHVVANPQAEGQLQWLNRRANALLANGVELRDNQLVVPSEGLYLIYSQVLFKGQGCPSTHVLLTHTISRIAVSYQTKVNLLSAIKSPCQRETPEGAEAKPWYEPIYLGGVFQLEKGDRLSAEINRPDYLNFRESGQVYFGIIAL

SEQ ID NO: 69 - protein, 489 aa, synthetic construct
  REGION 1..489: note = scTNFR2 (138)
METDTLLLWVLLLWVPGSTGMCGSHHHHHHSGIPAPVAHVVANPQAEGQLQWLNRRANALLANGVELRDNQLVVPSEGLYLIYSQVLFKGQGCPSTHVLLTHTISRIAVSYQTKVNLLSAIKSPCQRETPEGAEAKPWYEPIYLGGVFQLEKGDRLSAEINRPDYLNFRESGQVYFGIIALGGGSGGGSPVAHVVANPQAEGQLQWLNRRANALLANGVELRDNQLVVPSEGLYLIYSQVLFKGQGCPSTHVLLTHTISRIAVSYQTKVNLLSAIKSPCQRETPEGAEAKPWYEPIYLGGVFQLEKGDRLSAEINRPDYLNFRESGQVYFGIIALGGGSGGGSPVAHVVANPQAEGQLQWLNRRANALLANGVELRDNQLVVPSEGLYLIYSQVLFKGQGCPSTHVLLTHTISRIAVSYQTKVNLLSAIKSPCQRETPEGAEAKPWYEPIYLGGVFQLEKGDRLSAEINRPDYLNFRESGQVYFGIIAL

SEQ ID NO: 70 - protein, 491 aa, synthetic construct
  REGION 1..491: note = scTNFR2 (130)
METDTLLLWVLLLWVPGSTGMCGSHHHHHHSGIPARTPSDKPVAHVVANPQAEGQLQWLNRRANALLANGVELRDNQLVVPSEGLYLIYSQVLFKGQGCPSTHVLLTHTISRIAVSYQTKVNLLSAIKSPCQRETPEGAEAKPWYEPIYLGGVFQLEKGDRLSAEINRPDYLNFRESGQVYFGIIALRTPSDKPVAHVVANPQAEGQLQWLNRRANALLANGVELRDNQLVVPSEGLYLIYSQVLFKGQGCPSTHVLLTHTISRIAVSYQTKVNLLSAIKSPCQRETPEGAEAKPWYEPIYLGGVFQLEKGDRLSAEINRPDYLNFRESGQVYFGIIALRTPSDKPVAHVVANPQAEGQLQWLNRRANALLANGVELRDNQLVVPSEGLYLIYSQVLFKGQGCPSTHVLLTHTISRIAVSYQTKVNLLSAIKSPCQRETPEGAEAKPWYEPIYLGGVFQLEKGDRLSAEINRPDYLNFRESGQVYFGIIAL

SEQ ID NO: 71 - protein, 479 aa, synthetic construct
  REGION 1..479: note = scTNFR2 (131)
METDTLLLWVLLLWVPGSTGMCGSHHHHHHSGIPADKPVAHVVANPQAEGQLQWLNRRANALLANGVELRDNQLVVPSEGLYLIYSQVLFKGQGCPSTHVLLTHTISRIAVSYQTKVNLLSAIKSPCQRETPEGAEAKPWYEPIYLGGVFQLEKGDRLSAEINRPDYLNFRESGQVYFGIIALDKPVAHVVANPQAEGQLQWLNRRANALLANGVELRDNQLVVPSEGLYLIYSQVLFKGQGCPSTHVLLTHTISRIAVSYQTKVNLLSAIKSPCQRETPEGAEAKPWYEPIYLGGVFQLEKGDRLSAEINRPDYLNFRESGQVYFGIIALDKPVAHVVANPQAEGQLQWLNRRANALLANGVELRDNQLVVPSEGLYLIYSQVLFKGQGCPSTHVLLTHTISRIAVSYQTKVNLLSAIKSPCQRETPEGAEAKPWYEPIYLGGVFQLEKGDRLSAEINRPDYLNFRESGQVYFGIIAL

SEQ ID NO: 72 - protein, 728 aa, synthetic construct
  REGION 1..728: note = scTNFR2(118)-Fc(dab) 745
METDTLLLWVLLLWVPGSTGSSRTPSDKPVAHVVANPQAEGQLQWLNRRANALLANGVELRDNQLVVPSEGLYLIYSQVLFKGQGCPSTHVLLTHTISRIAVSYQTKVNLLSAIKSPCQRETPEGAEAKPWYEPIYLGGVFQLEKGDRLSAEINRPDYLNFRESGQVYFGIIALGGGGSSSRTPSDKPVAHVVANPQAEGQLQWLNRRANALLANGVELRDNQLVVPSEGLYLIYSQVLFKGQGCPSTHVLLTHTISRIAVSYQTKVNLLSAIKSPCQRETPEGAEAKPWYEPIYLGGVFQLEKGDRLSAEINRPDYLNFRESGQVYFGIIALGGGGSSSRTPSDKPVAHVVANPQAEGQLQWLNRRANALLANGVELRDNQLVVPSEGLYLIYSQVLFKGQGCPSTHVLLTHTISRIAVSYQTKVNLLSAIKSPCQRETPEGAEAKPWYEPIYLGGVFQLEKGDRLSAEINRPDYLNFRESGQVYFGIIALGGSGGGGSGGDKTHTCPPCPAPPVAGPSVFLFPPKPKDTLMISRTPEVTCVVVDVSHEDPEVKFNWYVDGVEVHNAKTKPREEQYNSTYRVVSVLTVLHQDWLNGKEYKCKVSNKGLPSSIEKTISKAKGQPREPQVYTLPPSRDELTKNQVSLTCLVKGFYPSDIAVEWESNGQPENNYKTTPPVLDSDGSFFLYSKLTVDKSRWQQGNVFSCSVMHEALHNHYTQKSLSLSPGK

SEQ ID NO: 73 - protein, 718 aa, synthetic construct
  REGION 1..718: note = scTNFR2(127)-Fc(dab) 742
METDTLLLWVLLLWVPGSTGSSRTPSDKPVAHVVANPQAEGQLQWLNRRANALLANGVELRDNQLVVPSEGLYLIYSQVLFKGQGCPSTHVLLTHTISRIAVSYQTKVNLLSAIKSPCQRETPEGAEAKPWYEPIYLGGVFQLEKGDRLSAEINRPDYLNFRESGQVYFGIIALSSRTPSDKPVAHVVANPQAEGQLQWLNRRANALLANGVELRDNQLVVPSEGLYLIYSQVLFKGQGCPSTHVLLTHTISRIAVSYQTKVNLLSAIKSPCQRETPEGAEAKPWYEPIYLGGVFQLEKGDRLSAEINRPDYLNFRESGQVYFGIIALSSRTPSDKPVAHVVANPQAEGQLQWLNRRANALLANGVELRDNQLVVPSEGLYLIYSQVLFKGQGCPSTHVLLTHTISRIAVSYQTKVNLLSAIKSPCQRETPEGAEAKPWYEPIYLGGVFQLEKGDRLSAEINRPDYLNFRESGQVYFGIIALGGSGGGGSGGDKTHTCPPCPAPPVAGPSVFLFPPKPKDTLMISRTPEVTCVVVDVSHEDPEVKFNWYVDGVEVHNAKTKPREEQYNSTYRVVSVLTVLHQDWLNGKEYKCKVSNKGLPSSIEKTISKAKGQPREPQVYTLPPSRDELTKNQVSLTCLVKGFYPSDIAVEWESNGQPENNYKTTPPVLDSDGSFFLYSKLTVDKSRWQQGNVFSCSVMHEALHNHYTQKSLSLSPGK

SEQ ID NO: 74 - protein, 706 aa, synthetic construct
  REGION 1..706: note = scTNFR2(129)-Fc(dab) 743
METDTLLLWVLLLWVPGSTGPSDKPVAHVVANPQAEGQLQWLNRRANALLANGVELRDNQLVVPSEGLYLIYSQVLFKGQGCPSTHVLLTHTISRIAVSYQTKVNLLSAIKSPCQRETPEGAEAKPWYEPIYLGGVFQLEKGDRLSAEINRPDYLNFRESGQVYFGIIALPSDKPVAHVVANPQAEGQLQWLNRRANALLANGVELRDNQLVVPSEGLYLIYSQVLFKGQGCPSTHVLLTHTISRIAVSYQTKVNLLSAIKSPCQRETPEGAEAKPWYEPIYLGGVFQLEKGDRLSAEINRPDYLNFRESGQVYFGIIALPSDKPVAHVVANPQAEGQLQWLNRRANALLANGVELRDNQLVVPSEGLYLIYSQVLFKGQGCPSTHVLLTHTISRIAVSYQTKVNLLSAIKSPCQRETPEGAEAKPWYEPIYLGGVFQLEKGDRLSAEINRPDYLNFRESGQVYFGIIALGGSGGGGSGGDKTHTCPPCPAPPVAGPSVFLFPPKPKDTLMISRTPEVTCVVVDVSHEDPEVKFNWYVDGVEVHNAKTKPREEQYNSTYRVVSVLTVLHQDWLNGKEYKCKVSNKGLPSSIEKTISKAKGQPREPQVYTLPPSRDELTKNQVSLTCLVKGFYPSDIAVEWESNGQPENNYKTTPPVLDSDGSFFLYSKLTVDKSRWQQGNVFSCSVMHEALHNHYTQKSLSLSPGK

SEQ ID NO: 75 - protein, 711 aa, synthetic construct
  REGION 1..711: note = scTNFR2(139)-Fc(dab) 744
METDTLLLWVLLLWVPGSTGSDKPVAHVVANPQAEGQLQWLNRRANALLANGVELRDNQLVVPSEGLYLIYSQVLFKGQGCPSTHVLLTHTISRIAVSYQTKVNLLSAIKSPCQRETPEGAEAKPWYEPIYLGGVFQLEKGDRLSAEINRPDYLNFRESGQVYFGIIALGGGGSDKPVAHVVANPQAEGQLQWLNRRANALLANGVELRDNQLVVPSEGLYLIYSQVLFKGQGCPSTHVLLTHTISRIAVSYQTKVNLLSAIKSPCQRETPEGAEAKPWYEPIYLGGVFQLEKGDRLSAEINRPDYLNFRESGQVYFGIIALGGGGSDKPVAHVVANPQAEGQLQWLNRRANALLANGVELRDNQLVVPSEGLYLIYSQVLFKGQGCPSTHVLLTHTISRIAVSYQTKVNLLSAIKSPCQRETPEGAEAKPWYEPIYLGGVFQLEKGDRLSAEINRPDYLNFRESGQVYFGIIALGGSGGGGSGGDKTHTCPPCPAPPVAGPSVFLFPPKPKDTLMISRTPEVTCVVVDVSHEDPEVKFNWYVDGVEVHNAKTKPREEQYNSTYRVVSVLTVLHQDWLNGKEYKCKVSNKGLPSSIEKTISKAKGQPREPQVYTLPPSRDELTKNQVSLTCLVKGFYPSDIAVEWESNGQPENNYKTTPPVLDSDGSFFLYSKLTVDKSRWQQGNVFSCSVMHEALHNHYTQKSLSLSPGK

SEQ ID NO: 76 - protein, 495 aa, synthetic construct
  REGION 1..495: note = variant 140
METDTLLLWVLLLWVPGSTGMCGSHHHHHHSGIPASSRTPSDKPVAHVVANPQAEGQLQWLNRRANALLANGVELRDNQLVVPSEGLYLIYSQVLFKGQGCPSTHVLLTHTISRIAVSYQTKVNLLSAIKSPCQRETPEGAEAKPWYEPIYLGGVFQLEKGDRLSAEINRPDYLNFRESGQVYFGIIALSRTPSDKPVAHVVANPQAEGQLQWLNRRANALLANGVELRDNQLVVPSEGLYLIYSQVLFKGQGCPSTHVLLTHTISRIAVSYQTKVNLLSAIKSPCQRETPEGAEAKPWYEPIYLGGVFQLEKGDRLSAEINRPDYLNFRESGQVYFGIIALSRTPSDKPVAHVVANPQAEGQLQWLNRRANALLANGVELRDNQLVVPSEGLYLIYSQVLFKGQGCPSTHVLLTHTISRIAVSYQTKVNLLSAIKSPCQRETPEGAEAKPWYEPIYLGGVFQLEKGDRLSAEINRPDYLNFRESGQVYFGIIAL

SEQ ID NO: 77 - protein, 497 aa, synthetic construct
  REGION 1..497: note = variant 141
METDTLLLWVLLLWVPGSTGMCGSHHHHHHSGIPASSRTPSDKPVAHVVANPQAEGQLQWLNRRANALLANGVELRDNQLVVPSEGLYLIYSQVLFKGQGCPSTHVLLTHTISRIAVSYQTKVNLLSAIKSPCQRETPEGAEAKPWYEPIYLGGVFQLEKGDRLSAEINRPDYLNFRESGQVYFGIIALGSRTPSDKPVAHVVANPQAEGQLQWLNRRANALLANGVELRDNQLVVPSEGLYLIYSQVLFKGQGCPSTHVLLTHTISRIAVSYQTKVNLLSAIKSPCQRETPEGAEAKPWYEPIYLGGVFQLEKGDRLSAEINRPDYLNFRESGQVYFGIIALGSRTPSDKPVAHVVANPQAEGQLQWLNRRANALLANGVELRDNQLVVPSEGLYLIYSQVLFKGQGCPSTHVLLTHTISRIAVSYQTKVNLLSAIKSPCQRETPEGAEAKPWYEPIYLGGVFQLEKGDRLSAEINRPDYLNFRESGQVYFGIIAL

SEQ ID NO: 78 - protein, 495 aa, synthetic construct
  REGION 1..495: note = variant 142
METDTLLLWVLLLWVPGSTGMCGSHHHHHHSGIPASSRTPSDKPVAHVVANPQAEGQLQWLNRRANALLANGVELRDNQLVVPSEGLYLIYSQVLFKGQGCPSTHVLLTHTISRIAVSYQTKVNLLSAIKSPCQRETPEGAEAKPWYEPIYLGGVFQLEKGDRLSAEINRPDYLNFRESGQVYFGIIALGRTPSDKPVAHVVANPQAEGQLQWLNRRANALLANGVELRDNQLVVPSEGLYLIYSQVLFKGQGCPSTHVLLTHTISRIAVSYQTKVNLLSAIKSPCQRETPEGAEAKPWYEPIYLGGVFQLEKGDRLSAEINRPDYLNFRESGQVYFGIIALGRTPSDKPVAHVVANPQAEGQLQWLNRRANALLANGVELRDNQLVVPSEGLYLIYSQVLFKGQGCPSTHVLLTHTISRIAVSYQTKVNLLSAIKSPCQRETPEGAEAKPWYEPIYLGGVFQLEKGDRLSAEINRPDYLNFRESGQVYFGIIAL

SEQ ID NO: 79 - protein, 490 aa, synthetic construct
  REGION 1..490: note = variant 143
METDTLLLWVLLLWVPGSTGMCGSHHHHHHSGIPASDKPVAHVVANPQAEGQLQWLNRRANALLANGVELRDNQLVVPSEGLYLIYSQVLFKGQGCPSTHVLLTHTISRIAVSYQTKVNLLSAIKSPCQRETPEGAEAKPWYEPIYLGGVFQLEKGDRLSAEINRPDYLNFRESGQVYFGIIALGGGPSDKPVAHVVANPQAEGQLQWLNRRANALLANGVELRDNQLVVPSEGLYLIYSQVLFKGQGCPSTHVLLTHTISRIAVSYQTKVNLLSAIKSPCQRETPEGAEAKPWYEPIYLGGVFQLEKGDRLSAEINRPDYLNFRESGQVYFGIIALGGGPSDKPVAHVVANPQAEGQLQWLNRRANALLANGVELRDNQLVVPSEGLYLIYSQVLFKGQGCPSTHVLLTHTISRIAVSYQTKVNLLSAIKSPCQRETPEGAEAKPWYEPIYLGGVFQLEKGDRLSAEINRPDYLNFRESGQVYFGIIAL

SEQ ID NO: 80 - protein, 497 aa, synthetic construct
  REGION 1..497: note = variant 144
METDTLLLWVLLLWVPGSTGMCGSHHHHHHSGIPASSRTPSDKPVAHVVANPQAEGQLQWLNRRANALLANGVELRDNQLVVPSEGLYLIYSQVLFKGQGCPSTHVLLTHTISRIAVSYQTKVNLLSAIKSPCQRETPEGAEAKPWYEPIYLGGVFQLEKGDRLSAEINRPDYLNFRESGQVYFGIIALGGRTPSDKPVAHVVANPQAEGQLQWLNRRANALLANGVELRDNQLVVPSEGLYLIYSQVLFKGQGCPSTHVLLTHTISRIAVSYQTKVNLLSAIKSPCQRETPEGAEAKPWYEPIYLGGVFQLEKGDRLSAEINRPDYLNFRESGQVYFGIIALGGRTPSDKPVAHVVANPQAEGQLQWLNRRANALLANGVELRDNQLVVPSEGLYLIYSQVLFKGQGCPSTHVLLTHTISRIAVSYQTKVNLLSAIKSPCQRETPEGAEAKPWYEPIYLGGVFQLEKGDRLSAEINRPDYLNFRESGQVYFGIIAL

SEQ ID NO: 81 - protein, 493 aa, synthetic construct
  REGION 1..493: note = variant 145
METDTLLLWVLLLWVPGSTGMCGSHHHHHHSGIPARTPSDKPVAHVVANPQAEGQLQWLNRRANALLANGVELRDNQLVVPSEGLYLIYSQVLFKGQGCPSTHVLLTHTISRIAVSYQTKVNLLSAIKSPCQRETPEGAEAKPWYEPIYLGGVFQLEKGDRLSAEINRPDYLNFRESGQVYFGIIALGGTPSDKPVAHVVANPQAEGQLQWLNRRANALLANGVELRDNQLVVPSEGLYLIYSQVLFKGQGCPSTHVLLTHTISRIAVSYQTKVNLLSAIKSPCQRETPEGAEAKPWYEPIYLGGVFQLEKGDRLSAEINRPDYLNFRESGQVYFGIIALGGTPSDKPVAHVVANPQAEGQLQWLNRRANALLANGVELRDNQLVVPSEGLYLIYSQVLFKGQGCPSTHVLLTHTISRIAVSYQTKVNLLSAIKSPCQRETPEGAEAKPWYEPIYLGGVFQLEKGDRLSAEINRPDYLNFRESGQVYFGIIAL

SEQ ID NO: 82 - protein, 492 aa, synthetic construct
  REGION 1..492: note = variant 146
METDTLLLWVLLLWVPGSTGMCGSHHHHHHSGIPASDKPVAHVVANPQAEGQLQWLNRRANALLANGVELRDNQLVVPSEGLYLIYSQVLFKGQGCPSTHVLLTHTISRIAVSYQTKVNLLSAIKSPCQRETPEGAEAKPWYEPIYLGGVFQLEKGDRLSAEINRPDYLNFRESGQVYFGIIALGGGTPSDKPVAHVVANPQAEGQLQWLNRRANALLANGVELRDNQLVVPSEGLYLIYSQVLFKGQGCPSTHVLLTHTISRIAVSYQTKVNLLSAIKSPCQRETPEGAEAKPWYEPIYLGGVFQLEKGDRLSAEINRPDYLNFRESGQVYFGIIALGGGTPSDKPVAHVVANPQAEGQLQWLNRRANALLANGVELRDNQLVVPSEGLYLIYSQVLFKGQGCPSTHVLLTHTISRIAVSYQTKVNLLSAIKSPCQRETPEGAEAKPWYEPIYLGGVFQLEKGDRLSAEINRPDYLNFRESGQVYFGIIAL

SEQ ID NO: 83 - protein, 492 aa, synthetic construct
  REGION 1..492: note = variant 147
METDTLLLWVLLLWVPGSTGMCGSHHHHHHSGIPASDKPVAHVVANPQAEGQLQWLNRRANALLANGVELRDNQLVVPSEGLYLIYSQVLFKGQGCPSTHVLLTHTISRIAVSYQTKVNLLSAIKSPCQRETPEGAEAKPWYEPIYLGGVFQLEKGDRLSAEINRPDYLNFRESGQVYFGIIALGGGGPSDKPVAHVVANPQAEGQLQWLNRRANALLANGVELRDNQLVVPSEGLYLIYSQVLFKGQGCPSTHVLLTHTISRIAVSYQTKVNLLSAIKSPCQRETPEGAEAKPWYEPIYLGGVFQLEKGDRLSAEINRPDYLNFRESGQVYFGIIALGGGGPSDKPVAHVVANPQAEGQLQWLNRRANALLANGVELRDNQLVVPSEGLYLIYSQVLFKGQGCPSTHVLLTHTISRIAVSYQTKVNLLSAIKSPCQRETPEGAEAKPWYEPIYLGGVFQLEKGDRLSAEINRPDYLNFRESGQVYFGIIAL

SEQ ID NO: 84 - protein, 716 aa, synthetic construct
  REGION 1..716: note = variant 148
METDTLLLWVLLLWVPGSTGSSRTPSDKPVAHVVANPQAEGQLQWLNRRANALLANGVELRDNQLVVPSEGLYLIYSQVLFKGQGCPSTHVLLTHTISRIAVSYQTKVNLLSAIKSPCQRETPEGAEAKPWYEPIYLGGVFQLEKGDRLSAEINRPDYLNFRESGQVYFGIIALSRTPSDKPVAHVVANPQAEGQLQWLNRRANALLANGVELRDNQLVVPSEGLYLIYSQVLFKGQGCPSTHVLLTHTISRIAVSYQTKVNLLSAIKSPCQRETPEGAEAKPWYEPIYLGGVFQLEKGDRLSAEINRPDYLNFRESGQVYFGIIALSRTPSDKPVAHVVANPQAEGQLQWLNRRANALLANGVELRDNQLVVPSEGLYLIYSQVLFKGQGCPSTHVLLTHTISRIAVSYQTKVNLLSAIKSPCQRETPEGAEAKPWYEPIYLGGVFQLEKGDRLSAEINRPDYLNFRESGQVYFGIIALGGSGGGGSGGDKTHTCPPCPAPPVAGPSVFLFPPKPKDTLMISRTPEVTCVVVDVSHEDPEVKFNWYVDGVEVHNAKTKPREEQYNSTYRVVSVLTVLHQDWLNGKEYKCKVSNKGLPSSIEKTISKAKGQPREPQVYTLPPSRDELTKNQVSLTCLVKGFYPSDIAVEWESNGQPENNYKTTPPVLDSDGSFFLYSKLTVDKSRWQQGNVFSCSVMHEALHNHYTQKSLSLSPGK

SEQ ID NO: 85 - protein, 718 aa, synthetic construct
  REGION 1..718: note = variant 149
METDTLLLWVLLLWVPGSTGSSRTPSDKPVAHVVANPQAEGQLQWLNRRANALLANGVELRDNQLVVPSEGLYLIYSQVLFKGQGCPSTHVLLTHTISRIAVSYQTKVNLLSAIKSPCQRETPEGAEAKPWYEPIYLGGVFQLEKGDRLSAEINRPDYLNFRESGQVYFGIIALGSRTPSDKPVAHVVANPQAEGQLQWLNRRANALLANGVELRDNQLVVPSEGLYLIYSQVLFKGQGCPSTHVLLTHTISRIAVSYQTKVNLLSAIKSPCQRETPEGAEAKPWYEPIYLGGVFQLEKGDRLSAEINRPDYLNFRESGQVYFGIIALGSRTPSDKPVAHVVANPQAEGQLQWLNRRANALLANGVELRDNQLVVPSEGLYLIYSQVLFKGQGCPSTHVLLTHTISRIAVSYQTKVNLLSAIKSPCQRETPEGAEAKPWYEPIYLGGVFQLEKGDRLSAEINRPDYLNFRESGQVYFGIIALGGSGGGGSGGDKTHTCPPCPAPPVAGPSVFLFPPKPKDTLMISRTPEVTCVVVDVSHEDPEVKFNWYVDGVEVHNAKTKPREEQYNSTYRVVSVLTVLHQDWLNGKEYKCKVSNKGLPSSIEKTISKAKGQPREPQVYTLPPSRDELTKNQVSLTCLVKGFYPSDIAVEWESNGQPENNYKTTPPVLDSDGSFFLYSKLTVDKSRWQQGNVFSCSVMHEALHNHYTQKSLSLSPGK

SEQ ID NO: 86 - protein, 711 aa, synthetic construct
  REGION 1..711: note = variant 150
METDTLLLWVLLLWVPGSTGSDKPVAHVVANPQAEGQLQWLNRRANALLANGVELRDNQLVVPSEGLYLIYSQVLFKGQGCPSTHVLLTHTISRIAVSYQTKVNLLSAIKSPCQRETPEGAEAKPWYEPIYLGGVFQLEKGDRLSAEINRPDYLNFRESGQVYFGIIALGRTPSDKPVAHVVANPQAEGQLQWLNRRANALLANGVELRDNQLVVPSEGLYLIYSQVLFKGQGCPSTHVLLTHTISRIAVSYQTKVNLLSAIKSPCQRETPEGAEAKPWYEPIYLGGVFQLEKGDRLSAEINRPDYLNFRESGQVYFGIIALGRTPSDKPVAHVVANPQAEGQLQWLNRRANALLANGVELRDNQLVVPSEGLYLIYSQVLFKGQGCPSTHVLLTHTISRIAVSYQTKVNLLSAIKSPCQRETPEGAEAKPWYEPIYLGGVFQLEKGDRLSAEINRPDYLNFRESGQVYFGIIALGGSGGGGSGGDKTHTCPPCPAPPVAGPSVFLFPPKPKDTLMISRTPEVTCVVVDVSHEDPEVKFNWYVDGVEVHNAKTKPREEQYNSTYRVVSVLTVLHQDWLNGKEYKCKVSNKGLPSSIEKTISKAKGQPREPQVYTLPPSRDELTKNQVSLTCLVKGFYPSDIAVEWESNGQPENNYKTTPPVLDSDGSFFLYSKLTVDKSRWQQGNVFSCSVMHEALHNHYTQKSLSLSPGK

SEQ ID NO: 87 - protein, 711 aa, synthetic construct
  REGION 1..711: note = variant 151
METDTLLLWVLLLWVPGSTGSDKPVAHVVANPQAEGQLQWLNRRANALLANGVELRDNQLVVPSEGLYLIYSQVLFKGQGCPSTHVLLTHTISRIAVSYQTKVNLLSAIKSPCQRETPEGAEAKPWYEPIYLGGVFQLEKGDRLSAEINRPDYLNFRESGQVYFGIIALGGGPSDKPVAHVVANPQAEGQLQWLNRRANALLANGVELRDNQLVVPSEGLYLIYSQVLFKGQGCPSTHVLLTHTISRIAVSYQTKVNLLSAIKSPCQRETPEGAEAKPWYEPIYLGGVFQLEKGDRLSAEINRPDYLNFRESGQVYFGIIALGGGPSDKPVAHVVANPQAEGQLQWLNRRANALLANGVELRDNQLVVPSEGLYLIYSQVLFKGQGCPSTHVLLTHTISRIAVSYQTKVNLLSAIKSPCQRETPEGAEAKPWYEPIYLGGVFQLEKGDRLSAEINRPDYLNFRESGQVYFGIIALGGSGGGGSGGDKTHTCPPCPAPPVAGPSVFLFPPKPKDTLMISRTPEVTCVVVDVSHEDPEVKFNWYVDGVEVHNAKTKPREEQYNSTYRVVSVLTVLHQDWLNGKEYKCKVSNKGLPSSIEKTISKAKGQPREPQVYTLPPSRDELTKNQVSLTCLVKGFYPSDIAVEWESNGQPENNYKTTPPVLDSDGSFFLYSKLTVDKSRWQQGNVFSCSVMHEALHNHYTQKSLSLSPGK

SEQ ID NO: 88 - protein, 718 aa, synthetic construct
  REGION 1..718: note = variant 152
METDTLLLWVLLLWVPGSTGSSRTPSDKPVAHVVANPQAEGQLQWLNRRANALLANGVELRDNQLVVPSEGLYLIYSQVLFKGQGCPSTHVLLTHTISRIAVSYQTKVNLLSAIKSPCQRETPEGAEAKPWYEPIYLGGVFQLEKGDRLSAEINRPDYLNFRESGQVYFGIIALGGRTPSDKPVAHVVANPQAEGQLQWLNRRANALLANGVELRDNQLVVPSEGLYLIYSQVLFKGQGCPSTHVLLTHTISRIAVSYQTKVNLLSAIKSPCQRETPEGAEAKPWYEPIYLGGVFQLEKGDRLSAEINRPDYLNFRESGQVYFGIIALGGRTPSDKPVAHVVANPQAEGQLQWLNRRANALLANGVELRDNQLVVPSEGLYLIYSQVLFKGQGCPSTHVLLTHTISRIAVSYQTKVNLLSAIKSPCQRETPEGAEAKPWYEPIYLGGVFQLEKGDRLSAEINRPDYLNFRESGQVYFGIIALGGSGGGGSGGDKTHTCPPCPAPPVAGPSVFLFPPKPKDTLMISRTPEVTCVVVDVSHEDPEVKFNWYVDGVEVHNAKTKPREEQYNSTYRVVSVLTVLHQDWLNGKEYKCKVSNKGLPSSIEKTISKAKGQPREPQVYTLPPSRDELTKNQVSLTCLVKGFYPSDIAVEWESNGQPENNYKTTPPVLDSDGSFFLYSKLTVDKSRWQQGNVFSCSVMHEALHNHYTQKSLSLSPGK

SEQ ID NO: 89 - protein, 714 aa, synthetic construct
  REGION 1..714: note = variant 153
METDTLLLWVLLLWVPGSTGRTPSDKPVAHVVANPQAEGQLQWLNRRANALLANGVELRDNQLVVPSEGLYLIYSQVLFKGQGCPSTHVLLTHTISRIAVSYQTKVNLLSAIKSPCQRETPEGAEAKPWYEPIYLGGVFQLEKGDRLSAEINRPDYLNFRESGQVYFGIIALGGTPSDKPVAHVVANPQAEGQLQWLNRRANALLANGVELRDNQLVVPSEGLYLIYSQVLFKGQGCPSTHVLLTHTISRIAVSYQTKVNLLSAIKSPCQRETPEGAEAKPWYEPIYLGGVFQLEKGDRLSAEINRPDYLNFRESGQVYFGIIALGGTPSDKPVAHVVANPQAEGQLQWLNRRANALLANGVELRDNQLVVPSEGLYLIYSQVLFKGQGCPSTHVLLTHTISRIAVSYQTKVNLLSAIKSPCQRETPEGAEAKPWYEPIYLGGVFQLEKGDRLSAEINRPDYLNFRESGQVYFGIIALGGSGGGGSGGDKTHTCPPCPAPPVAGPSVFLFPPKPKDTLMISRTPEVTCVVVDVSHEDPEVKFNWYVDGVEVHNAKTKPREEQYNSTYRVVSVLTVLHQDWLNGKEYKCKVSNKGLPSSIEKTISKAKGQPREPQVYTLPPSRDELTKNQVSLTCLVKGFYPSDIAVEWESNGQPENNYKTTPPVLDSDGSFFLYSKLTVDKSRWQQGNVFSCSVMHEALHNHYTQKSLSLSPGK

SEQ ID NO: 90 - protein, 713 aa, synthetic construct
  REGION 1..713: note = variant 154
METDTLLLWVLLLWVPGSTGSDKPVAHVVANPQAEGQLQWLNRRANALLANGVELRDNQLVVPSEGLYLIYSQVLFKGQGCPSTHVLLTHTISRIAVSYQTKVNLLSAIKSPCQRETPEGAEAKPWYEPIYLGGVFQLEKGDRLSAEINRPDYLNFRESGQVYFGIIALGGGTPSDKPVAHVVANPQAEGQLQWLNRRANALLANGVELRDNQLVVPSEGLYLIYSQVLFKGQGCPSTHVLLTHTISRIAVSYQTKVNLLSAIKSPCQRETPEGAEAKPWYEPIYLGGVFQLEKGDRLSAEINRPDYLNFRESGQVYFGIIALGGGTPSDKPVAHVVANPQAEGQLQWLNRRANALLANGVELRDNQLVVPSEGLYLIYSQVLFKGQGCPSTHVLLTHTISRIAVSYQTKVNLLSAIKSPCQRETPEGAEAKPWYEPIYLGGVFQLEKGDRLSAEINRPDYLNFRESGQVYFGIIALGGSGGGGSGGDKTHTCPPCPAPPVAGPSVFLFPPKPKDTLMISRTPEVTCVVVDVSHEDPEVKFNWYVDGVEVHNAKTKPREEQYNSTYRVVSVLTVLHQDWLNGKEYKCKVSNKGLPSSIEKTISKAKGQPREPQVYTLPPSRDELTKNQVSLTCLVKGFYPSDIAVEWESNGQPENNYKTTPPVLDSDGSFFLYSKLTVDKSRWQQGNVFSCSVMHEALHNHYTQKSLSLSPGK

SEQ ID NO: 91 - protein, 713 aa, synthetic construct
  REGION 1..713: note = variant 155
METDTLLLWVLLLWVPGSTGSDKPVAHVVANPQAEGQLQWLNRRANALLANGVELRDNQLVVPSEGLYLIYSQVLFKGQGCPSTHVLLTHTISRIAVSYQTKVNLLSAIKSPCQRETPEGAEAKPWYEPIYLGGVFQLEKGDRLSAEINRPDYLNFRESGQVYFGIIALGGGGPSDKPVAHVVANPQAEGQLQWLNRRANALLANGVELRDNQLVVPSEGLYLIYSQVLFKGQGCPSTHVLLTHTISRIAVSYQTKVNLLSAIKSPCQRETPEGAEAKPWYEPIYLGGVFQLEKGDRLSAEINRPDYLNFRESGQVYFGIIALGGGGPSDKPVAHVVANPQAEGQLQWLNRRANALLANGVELRDNQLVVPSEGLYLIYSQVLFKGQGCPSTHVLLTHTISRIAVSYQTKVNLLSAIKSPCQRETPEGAEAKPWYEPIYLGGVFQLEKGDRLSAEINRPDYLNFRESGQVYFGIIALGGSGGGGSGGDKTHTCPPCPAPPVAGPSVFLFPPKPKDTLMISRTPEVTCVVVDVSHEDPEVKFNWYVDGVEVHNAKTKPREEQYNSTYRVVSVLTVLHQDWLNGKEYKCKVSNKGLPSSIEKTISKAKGQPREPQVYTLPPSRDELTKNQVSLTCLVKGFYPSDIAVEWESNGQPENNYKTTPPVLDSDGSFFLYSKLTVDKSRWQQGNVFSCSVMHEALHNHYTQKSLSLSPGK

SEQ ID NO: 92 - protein, 10 aa, synthetic construct
  REGION 1..10: note = linker
GGSGGGGSGG

SEQ ID NO: 93 - protein, 18 aa, synthetic construct
  REGION 1..18: note = from variant 141
GIIALGSRTPSDKPVAHV

SEQ ID NO: 94 - protein, 18 aa, synthetic construct
  REGION 1..18: note = from variant 144
GIIALGGRTPSDKPVAHV

SEQ ID NO: 95 - protein, 18 aa, synthetic construct
  REGION 1..18: note = from variant 146
GIIALGGGTPSDKPVAHV

SEQ ID NO: 96 - protein, 18 aa, synthetic construct
  REGION 1..18: note = from variant 147
GIIALGGGGPSDKPVAHV

SEQ ID NO: 97 - protein, 17 aa, synthetic construct
  REGION 1..17: note = from variant 140
GIIALSRTPSDKPVAHV

SEQ ID NO: 98 - protein, 17 aa, synthetic construct
  REGION 1..17: note = from variant 142
GIIALGRTPSDKPVAHV

SEQ ID NO: 99 - protein, 17 aa, synthetic construct
  REGION 1..17: note = from variant 145
GIIALGGTPSDKPVAHV

SEQ ID NO: 100 - protein, 17 aa, synthetic construct
  REGION 1..17: note = from variant 143
GIIALGGGPSDKPVAHV

SEQ ID NO: 101 - protein, 18 aa, synthetic construct
  REGION 1..18: note = from variant 149
GIIALGSRTPSDKPVAHV

SEQ ID NO: 102 - protein, 18 aa, synthetic construct
  REGION 1..18: note = from variant 152
GIIALGGRTPSDKPVAHV

SEQ ID NO: 103 - protein, 18 aa, synthetic construct
  REGION 1..18: note = from variant 154
GIIALGGGTPSDKPVAHV

SEQ ID NO: 104 - protein, 18 aa, synthetic construct
  REGION 1..18: note = from variant 155
GIIALGGGGPSDKPVAHV

SEQ ID NO: 105 - protein, 17 aa, synthetic construct
  REGION 1..17: note = from variant 148
GIIALSRTPSDKPVAHV

SEQ ID NO: 106 - protein, 17 aa, synthetic construct
  REGION 1..17: note = from variant 150
GIIALGRTPSDKPVAHV

SEQ ID NO: 107 - protein, 17 aa, synthetic construct
  REGION 1..17: note = from variant 153
GIIALGGTPSDKPVAHV

SEQ ID NO: 108 - protein, 17 aa, synthetic construct
  REGION 1..17: note = from variant 151
GIIALGGGPSDKPVAHV